European Patent Specification EP 4 083 073 B1, published April 9, 2025. Title: Novel Chimeric Antigen Receptor and Use thereof. Applicant: NANJING BIOHENG BIOTECH CO., LTD. The sequence listing filed with the application follows.

SEQUENCE LISTING (16 sequences)

SEQ ID NO: 1 - DNA, 726 bp, Artificial Sequence
  CD19 scFv
gacatccagatgacacagactacatcctccctgtctgcctctctgggagacagagtcaccatcagttgcagggcaagtcaggacattagtaaatatttaaattggtatcagcagaaaccagatggaactgttaaactcctgatctaccatacatcaagattacactcaggagtcccatcaaggttcagtggcagtgggtctggaacagattattctctcaccattagcaacctggagcaagaagatattgccacttacttttgccaacagggtaatacgcttccgtacacgttcggaggggggaccaagctggagatcacaggtggcggtggctcgggcggtggtgggtcgggtggcggcggatctgaggtgaaactgcaggagtcaggacctggcctggtggcgccctcacagagcctgtccgtcacatgcactgtctcaggggtctcattacccgactatggtgtaagctggattcgccagcctccacgaaagggtctggagtggctgggagtaatatggggtagtgaaaccacatactataattcagctctcaaatccagactgaccatcatcaaggacaactccaagagccaagttttcttaaaaatgaacagtctgcaaactgatgacacagccatttactactgtgccaaacattattactacggtggtagctatgctatggactactggggccaaggaacctcagtcaccgtctcctca

SEQ ID NO: 2 - protein, 242 aa, Artificial Sequence
  CD19 scFv
DIQMTQTTSSLSASLGDRVTISCRASQDISKYLNWYQQKPDGTVKLLIYHTSRLHSGVPSRFSGSGSGTDYSLTISNLEQEDIATYFCQQGNTLPYTFGGGTKLEITGGGGSGGGGSGGGGSEVKLQESGPGLVAPSQSLSVTCTVSGVSLPDYGVSWIRQPPRKGLEWLGVIWGSETTYYNSALKSRLTIIKDNSKSQVFLKMNSLQTDDTAIYYCAKHYYYGGSYAMDYWGQGTSVTVSS

SEQ ID NO: 3 - DNA, 75 bp, Artificial Sequence
  CD8αtransmembrane domain
atctacatctgggcgcccttggccgggacttgtggggtccttctcctgtcactggttatcaccctttactgcaaa

SEQ ID NO: 4 - protein, 25 aa, Artificial Sequence
  CD8αtransmembrane domain
IYIWAPLAGTCGVLLLSLVITLYCK

SEQ ID NO: 5 - DNA, 120 bp, Artificial Sequence
  4-1BB co-stimulatory domain
cggggcagaaagaaactcctgtatatattcaaacaaccatttatgagaccagtacaaactactcaagaggaagatggctgtagctgccgatttccagaagaagaagaaggaggatgtgaa

SEQ ID NO: 6 - protein, 40 aa, Artificial Sequence
  4-1BB co-stimulatory domain
RGRKKLLYIFKQPFMRPVQTTQEEDGCSCRFPEEEEGGCE

SEQ ID NO: 7 - DNA, 339 bp, Artificial Sequence
  CD3ζsignaling domain
ctgagagtgaagttcagcaggagcgcagacgcccccgcgtaccagcagggccagaaccagctctataacgagctcaatctaggacgaagagaggagtacgatgttttggacaagagacgtggccgggaccctgagatggggggaaagccgagaaggaagaaccctcaggaaggcctgtacaatgaactgcagaaagataagatggcggaggcctacagtgagattgggatgaaaggcgagcgccggaggggcaaggggcacgatggcctttaccagggtctcagtacagccaccaaggacacctacgacgcccttcacatgcaggccctgccccctcgc

SEQ ID NO: 8 - protein, 113 aa, Artificial Sequence
  CD3ζsignaling domain
LRVKFSRSADAPAYQQGQNQLYNELNLGRREEYDVLDKRRGRDPEMGGKPRRKNPQEGLYNELQKDKMAEAYSEIGMKGERRRGKGHDGLYQGLSTATKDTYDALHMQALPPR

SEQ ID NO: 9 - DNA, 63 bp, Artificial Sequence
  CD8αsignal peptide
atggccttaccagtgaccgccttgctcctgccgctggccttgctgctccacgccgccaggccg

SEQ ID NO: 10 - protein, 21 aa, Artificial Sequence
  CD8αsignal peptide
MALPVTALLLPLALLLHAARP

SEQ ID NO: 11 - DNA, 135 bp, Artificial Sequence
  CD8αhinge region
accacgacgccagcgccgcgaccaccaacaccggcgcccaccatcgcgtcgcagcccctgtccctgcgcccagaggcgtgccggccagcggcggggggcgcagtgcacacgagggggctggacttcgcctgtgat

SEQ ID NO: 12 - protein, 45 aa, Artificial Sequence
  CD8αhinge region
TTTPAPRPPTPAPTIASQPLSLRPEACRPAAGGAVHTRGLDFACD

SEQ ID NO: 13 - DNA, 1107 bp, Artificial Sequence
  γc chain
atgttgaagccatcattaccattcacatccctcttattcctgcagctgcccctgctgggagtggggctgaacacgacaattctgacgcccaatgggaatgaagacaccacagctgatttcttcctgaccactatgcccactgactccctcagtgtttccactctgcccctcccagaggttcagtgttttgtgttcaatgtcgagtacatgaattgcacttggaacagcagctctgagccccagcctaccaacctcactctgcattattggtacaagaactcggataatgataaagtccagaagtgcagccactatctattctctgaagaaatcacttctggctgtcagttgcaaaaaaaggagatccacctctaccaaacatttgttgttcagctccaggacccacgggaacccaggagacaggccacacagatgctaaaactgcagaatctggtgatcccctgggctccagagaacctaacacttcacaaactgagtgaatcccagctagaactgaactggaacaacagattcttgaaccactgtttggagcacttggtgcagtaccggactgactgggaccacagctggactgaacaatcagtggattatagacataagttctccttgcctagtgtggatgggcagaaacgctacacgtttcgtgttcggagccgctttaacccactctgtggaagtgctcagcattggagtgaatggagccacccaatccactgggggagcaatacttcaaaagagaatcctttcctgtttgcattggaagccgtggttatctctgttggctccatgggattgattatcagccttctctgtgtgtatttctggctggaacggacgatgccccgaattcccaccctgaagaacctagaggatcttgttactgaataccacgggaacttttcggcctggagtggtgtgtctaagggactggctgagagtctgcagccagactacagtgaacgactctgcctcgtcagtgagattcccccaaaaggaggggcccttggggaggggcctggggcctccccatgcaaccagcatagcccctactgggcccccccatgttacaccctaaagcctgaaacc

SEQ ID NO: 14 - protein, 369 aa, Artificial Sequence
  γc chain
MLKPSLPFTSLLFLQLPLLGVGLNTTILTPNGNEDTTADFFLTTMPTDSLSVSTLPLPEVQCFVFNVEYMNCTWNSSSEPQPTNLTLHYWYKNSDNDKVQKCSHYLFSEEITSGCQLQKKEIHLYQTFVVQLQDPREPRRQATQMLKLQNLVIPWAPENLTLHKLSESQLELNWNNRFLNHCLEHLVQYRTDWDHSWTEQSVDYRHKFSLPSVDGQKRYTFRVRSRFNPLCGSAQHWSEWSHPIHWGSNTSKENPFLFALEAVVISVGSMGLIISLLCVYFWLERTMPRIPTLKNLEDLVTEYHGNFSAWSGVSKGLAESLQPDYSERLCLVSEIPPKGGALGEGPGASPCNQHSPYWAPPCYTLKPET

SEQ ID NO: 15 - DNA, 258 bp, Artificial Sequence
  γc chain intracellular region
gaacggacgatgccccgaattcccaccctgaagaacctagaggatcttgttactgaataccacgggaacttttcggcctggagtggtgtgtctaagggactggctgagagtctgcagccagactacagtgaacgactctgcctcgtcagtgagattcccccaaaaggaggggcccttggggaggggcctggggcctccccatgcaaccagcatagcccctactgggcccccccatgttacaccctaaagcctgaaacc

SEQ ID NO: 16 - protein, 86 aa, Artificial Sequence
  γc chain intracellular region
ERTMPRIPTLKNLEDLVTEYHGNFSAWSGVSKGLAESLQPDYSERLCLVSEIPPKGGALGEGPGASPCNQHSPYWAPPCYTLKPET